European Patent Specification EP 3 863 401 B1, published December 4, 2024. Title: Genetically modified Avians and Method for the Reconstitution Thereof. Applicant: The University Court of the University of Edinburgh. The sequence listing filed with the application follows.

SEQUENCE LISTING (18 sequences)

SEQ ID NO: 1 - DNA, 1317 bp, Artificial Sequence
  2a-iCaspase9-Bam H1 site mutated
ggatccggagctactaacttcagcctgctgaagcaggctggagacgtggaggagaaccctggacctatgctcgagggagtgcaggtggagactatctccccaggagacgggcgcaccttccccaagcgcggccagacctgcgtggtgcactacaccgggatgcttgaagatggaaagaaagttgattcctcccgggacagaaacaagccctttaagtttatgctaggcaagcaggaggtgatccgaggctgggaagaaggggttgcccagatgagtgtgggtcagagagccaaactgactatatctccagattatgcctatggtgccactgggcacccaggcatcatcccaccacatgccactctcgtcttcgatgtggagcttctaaaactggaatctggcggtggttccggagtcgacggatttggtgatgtcggtgctcttgagagtttgaggggaaatgcagatttggcttacatcctgagcatggagccctgtggccactgcctcattatcaacaatgtgaacttctgccgtgagtccgggctccgcacccgcactggctccaacatcgactgtgagaagttgcggcgtcgcttctcctcgctgcatttcatggtggaggtgaagggcgacctgactgccaagaaaatggtgctggctttgctggagctggcgcggcaggaccacggtgctctggactgctgcgtggtggtcattctctctcacggctgtcaggccagccacctgcagttcccaggggctgtctacggcacagatggatgccctgtgtcggtcgagaagattgtgaacatcttcaatgggaccagctgccccagcctgggagggaagcccaagctctttttcatccaggcctgtggtggggagcagaaagaccatgggtttgaggtggcctccacttcccctgaagacgagtcccctggcagtaaccccgagccagatgccaccccgttccaggaaggtttgaggaccttcgaccagctggacgccatatctagtttgcccacacccagtgacatctttgtgtcctactctactttcccaggttttgtttcctggagggaccccaagagtggctcctggtacgttgagaccctggacgacatctttgagcagtgggctcactctgaagacctgcagtccctcctgcttagggtcgctaatgctgtttcggtgaaagggatttataaacagatgcctggttgctttaatttcctccggaaaaaacttttctttaaaacatcagtcgactatccgtacgacgtaccagactacgcactcgacctcgacggatcc

SEQ ID NO: 2 - DNA, 1315 bp, Artificial Sequence
  2a-aviCaspase9
agggatccggagctactaacttcagcctgctgaagcaggctggagacgtggaggagaaccctggacctatgctcgagggagtgcaggtggagactatctccccaggagacgggcgcaccttccccaagcgcggccagacctgcgtggtgcactacaccgggatgcttgaagatggaaagaaagttgattcctcccgggacagaaacaagccctttaagtttatgcttggcaagcaggaggtgatccgaggctgggaagaaggggttgcccagatgagtgtgggtcagagagccaaactgactatatctccagattatgcctatggtgccactgggcacccaggcatcatcccaccacatgccactctcgtcttcgatgtggagcttctaaaactggaatctggcggtggttccggagtcgacggtgtctctgtgaattgcagaccagctaggatgcatgctagtgcatgccaggtgtaccagctgcgagcagacccttgtgggcactgcctgatcttcaacaatgtcagcttcagcagagactctgatctgtcgactcgagctggctctgacatagactgtgagaagctggagaagcgtttcaggtccctgtgcttccacgtccggaccctgcggaacctcaaagctcaggaaattgatgtggagctgcggaagctggcgcggctcgaccacagtgccctggactgctgcctcgtggtcatcctctcccatggttgccagacaagccatattcagtttcccggagggatttatggaacagatggcaaaatcattccaatcgaaaggattgtgaactatttcaatgggtcccagtgcccgagtttgagaggaaaacccaaactcttcttcatccaggcctgtggaggagaacaaaaggaccaaggatttgaggtggattgtgaatcaccccaagatgaaacttgccgacgttccatagagtcggatgcgattcctttccaggctccatcagggaatgaggacgagccagacgccgtcgccagtttgcccactcctggtgacatcttggtgtcctattcaacttttccaggttttgtgtcctggagggacaaggtgagtggctcgtggtacgtggaaaccttggacagcgtactggaacattacgcccgttctgaagacctgcttaccatgctacttcgggtgtcagacatcgtatccaccaaggggaggtacaagcagatcccgggctgtttcaacttccttcgtaaaaaattcttcttcctgtgcaaggtcgactatccgtacgacgtaccagactacgcactcgacggatccaa

SEQ ID NO: 3 - DNA, 5985 bp, Artificial Sequence
  Leftarm-GFP-2a-Nitroreductase-T2a-Right arm
tttttttctttgagatgagtatcttattgcagctctgtgcataccccttgaaaatccgtaggtgatgtatttatgttgactgaaaatggagtcattcaaaaattgatgacttcttccttttctctttttaatctcgaaacctgttctcagattcctttatcagaacaaaaagcacggctgcatgtttttcaccgttcacacgactgtgtttagccagcgtatctaaatgcataacatgatttgccataacttgagcctgccataatcagagcctcattttgaaagctgtcatggtctgaaacatagcatgggtaagatgattttcaccttgatgatgcatgtttaactcatttcaacgagaggtcaaatccatccaaaaatgctaaatctatcaaccagttttcatgttcaagttctggcacaaattttcgttctgactccatacgtgattagatttcattttgcaaatcatgaaaactattgccaaaacatacaattttaagtcagcagttttactgcccaaatttgcacaagcacatgtaacgtgacagacaaaaacccactggacagagacaaaatactgggtttggccagtatggtttggctaagccacgtttttcagggcaagaattgcctcacctttttttatattggaatcaaattctcaagtgtaacagcctggcgccatctcagctgccattaagtagcatgtgctgcaacaagatgtctaccacacactctgctctgggtggtgggggcacaccagtgtggacggcaaccatgacacaagcatagagtcttggcagaggtccattgggtgcatttatagtggttcacactggggggttatcacagaatcatggaggttggaaggtacctccgggggtcatcaaatccaaccacttgacaaagcaggttccctaaagtagattgctcaagaacagtcacagcactgctgctcacagaaaatctctagttggtaaggttacctttttttttgttgtcgctcccagttaaaccaaggtgggaacacatccttttcatagttgtattgtagggatgtttatagctattgctagggaaaactgaacagcgtgcaaggaagtcagcactgacacagctttcccacgtgagagagctatttcaaagcaagatcagcacatatcccaatctgtacttcctcaaacacagcccaaaaccgatagcaaggccaagcagcagcactgctccttcaaggaaactgctgcataatctgaatttcagacggcaggaggaaacaaggcagcagactgatgacctaccaccctgagtctcagctacatgcgatccgagccactccaactctgcttcctgcagcccttccttcacgctcatcttttgcaccttaggcactcttataattcaagtactttgtggctttgggatatttgaagagcttggtcagttagtcacaagtctggccacgtgctatcatattagtttgaaaagcaatggagacaccatctgctgatgctcaaagtggttacaaccaaaacacaaaaaagcagagctgtgggaagaattcaacattttgattatgcaagaagctagtcccagccttgaaatccaccatctgcatcatgaaagacctaagtagttaaagccacagcagacatacagcttctatttccttaccttcttcatcattaactacaggtcttggaagatttttgctgggaaaaagcttttattgcaagaactgtaatttattaacagggaaacatgaaataaatgtgtaaattctcctgcactcccactgtcattaaaaacggctttaagaaagagtattcagtaactgcctgcattgtgttgtgactttctactctgtgacacacagccttctgggcaaagcacatattctgccatgcatgtgggtcgtgccttggaaaatgggaacccacattcactgagggcctcttgatgagctttccccttgagaacagcgaggtctcatggatatcttctcttctccaagccaaataagcccagatccctcagctttccttcatggagaggctccagccctctgatcatgcctgcagcccttctctggacctgctccagcagccccacacgctcctcatgctgggaccccagatctgcacatggtattgcacatggggcctcacaacggcagagctgagagggacaattccctccctcagcctttaattctgcacgtacttaattttgtctgtattttttttgcaatagaatagcctgcatgctagttgctgtgtcgcacagctgaattcactaggttcctgtgaaacaaagggcaatcccacagccactgtagcacgtgaggagccacacaggtgctctaattcctacaggacaggcctagggacagagcggccctaggactgccctcccgcacctcctagcttcaccttttgcccgcgatctttaagtaccctgaagcataaacagggaaagcgccgcccgcagcctcaccctgcttcccgcccaacgcggcaccgcccaggccgcagccgcccactaagagcactagcgccaccttctcaccccacccccaccacgcgttcctagcggccctgagagctgctgcgcatgcgccgcctgacgattcgccctcccattggctggcggtcgaagcacggcgggggcacgcggtggcggctatataaggcgtctcggaagacggcgccatgctatttggagcggagagtgaaagttacagttcctggtgctggtagggagtgtggcgcggagcggagcgctgcggctcatcggaaccacaatggagccatagcagagccgggcgtgggggcaagggcagtgcgtgctggggagggctccgtcgcgtggccacgtcgcgagagccgtcgggatggtggcgtcagggcggggggtgctgctaacgtgctcctggtcctgcaggtgggctgctggcattcgccatggtgagcaagggcgaggagctgttcaccggggtggtgcccatcctggtcgagctggacggcgacgtaaacggccacaagttcagcgtgtccggcgagggcgagggcgatgccacctacggcaagctgaccctgaagttcatctgcaccaccggcaagctgcccgtgccctggcccaccctcgtgaccaccctgacctacggcgtgcagtgcttcagccgctaccccgaccacatgaagcagcacgacttcttcaagtccgccatgcccgaaggctacgtccaggagcgcaccatcttcttcaaggacgacggcaactacaagacccgcgccgaggtgaagttcgagggcgacaccctggtgaaccgcatcgagctgaagggcatcgacttcaaggaggacggcaacatcctggggcacaagctggagtacaactacaacagccacaacgtctatatcatggccgacaagcagaagaacggcatcaaggtgaacttcaagatccgccacaacatcgaggacggcagcgtgcagctcgccgaccactaccagcagaacacccccatcggcgacggccccgtgctgctgcccgacaaccactacctgagcacccagtccgccctgagcaaagaccccaacgagaagcgcgatcacatggtcctgctggagttcgtgaccgccgccgggatcactctcggcatggacgagctgtacaagggatccggagctactaacttcagcctgctgaagcaggctggagacgtggaggagaaccctggacctatggatatcatcagcgtggccctgaagagacacagcaccaaggccttcgatgccagcaagaagctgacccccgagcaggccgagcagatcaagaccctgctgcagtacagccccagcagccagaacagccagccctggcacttcatcgtggccagcaccgaggaaggcaaggccagagtggccaagagcgccgccggcaactacgtgttcagcgagagaaagatgctggatgccagccacgtggtggtgttctgcgccaagaccgctatggatgatgtgtggctgaagctggtggtggatcaggaggatgccgatggcagattcgccacccccgaggccaaggccgccaacgataagggcagaaagttcaccgccgatatgcacagaaaggatctgcacgatgatgccgagtggatggccaagcaggtgtacctgaacgtgggcaacttcctgctcggcgtggccgccctgggcctggatgccgtgcccatcgagggcttcgatgccgccatcctggatgccgagttcggcctgaaggagaagggctacaccagcctggtggtggtgcccgtgggccaccacagcgtggaggatttcaacgccaccctccccaagagcagactgccccagaacatcaccctgaccgaggtgggatccggagagggcagaggaagtctgctaacatgcggtgacgtcgaggagaatcctggacctatggaggaggattgggataccgaactcgagcaggaggcggcagcggcttcccaggggcgttctgaggagcaggcgtggatggtgagctgtgtccaggggagggcggtgcggcagggagcggggcactgggatggcccggtctgggaaggggaggccgagaggccttcgcagtgcttcctgcagctccccgagcagtgcgaagaaggaggtgccgggctctgctgtgggagccgaaggcacggagctgcctggggagggaatggctgtgtgcctgaggtgccagagaccggcaagggctgtacagagaggcaacggttttgtgtacaaatcatttgtatgggaaaccacaaaatcttgaagctttattacatggcagcgaaatactttggtgtgaagtaaaggataagatagaggagtgtaatgagagacagctaaataatattttactacttgtgggatgagtgaatatcaggaggaactgctgtaaatttcaggaggacctgttgtgaatcttcagtagttggcgccgctcttacacatcttacagatgccccttgagcaaagggggataaggagagatgaacgggttatccaaacaggtgatgagctaaaagtacagttgcctaaagaagtagtagcatgtgctatcagaatgataattttgttagtttggggttagtttcctgtagtggtagatagccacaacaagaaaaccgcttaagtttttgtaaaacaaaaaaagcacgatccagaagtaaaaaatatgggtagttttttttgatgttcctctctcacctggtgctttggcatactaatatgtgtctaattgtattaaacaggagaaatttaaacctaggctttgctggaaataaaatgttacaatgctacaatgtgaaaagtaggtgctattctgaactgttttgggtggagtatctgaatctttgaataatttaagagggactgacatatttaaaatacttaaggataatctgtagccatgctgtaaaagaacaacagaaatgcagttgggaaggtgatggaaatagttttattcatgttactggtggtctgaaacctttctaagcttaaactgtagaaaaaaattgcttcaaaagattgcactattactttgggcgacaaatgtttttaattggttttaagtgtttgttagcaaagtgaagttgatgccaccataagtctgacaggaggcaagataaacttgtcttcatactgcttgtgtataacttggttttgatgacatttgtgtgtgaacattatgcacttcagtgtagcgaagtttaagaaactttgaacagaataacttgaaagagtgtgcacatgggtgcagaagtcactttatttcagttgggagacttagcacctaaatgcactgttagttcacatacactttgcttggcctgaaggtaacattgtgatgtcgctttttttccctgtaggctaactctggcagaccaaacagcccatccctccgcttctccagcagaccaagcagccccttgtctgg

SEQ ID NO: 4 - DNA, 5155 bp, Artificial Sequence
  Left arm-2a-aviCaspase9-T2a-GFP-Right arm
cttcgtggcttggtgaagagatcttctgacctcttcatcaccccctagaattaaggctgtaatcatcatttcagccattgcttaatccactataatttctgcatgatttcagaaggctatcttgcttccttgaaactaataatacctagtttgtagtgtttagggatgtgtaaaatgtgtttatgtcaagattttagttagtctgataagaattgtggaagaattgcagctactaaaaaggcagactgggtagcacttcccaccttactcagatttaggagtctcaagacatgtagatgggtgaaatttattattcttttctctgcttgcttttctggaaagctacctctatttggccagcagttggctctgaattcctttctttaaaggagacctgactgctctcctgtctgcctcttacacagctgtactggtgtgtcactgatagaaacgtttaccttgaaagtgacaagtgggggcgttgatacccattaacaacattaaagggaaaatttcaggaaacaagaaaactgagaggagttcagaatgaaatgtaagccctgtgacagactcacactgatggtagtagggtaactgatggagatgcatctataacaattctaacttttatttcagaagtctgtggacaggagcatacaaacagtagtatcttgtctgtttaaccctgaaaaccgtctgaggaacacctttgtatcacaagaagactacttcagggtatgtagtgaaagcaaaactaaatctctaaaaccagctgatcttaactttgttcatatacaggatgccatgaagacaaaggtttatctgtacttgcttgagattttactttttgtatgtgcattgagatgaatgactggttagctctcagttggttaatactcaatgaaaattgcagaaattgagttcagtggatttaagtgcattgatacaaggctgcataagaactgctgagcagtcagctattggatatttagagctaatcatccctcaggagcaatctgctgaaaggtaagcagattgcatcttgtaaacgagagagcagagttaaacgtttgtggtctttgctccacttaagtacccacagtggatgtctatctgtacttttggttaaaaaatagataatttctacaacagactgtagttaggtcagtacctggtcatcaggtattaatggaaagctttttgctgtgcattcaatcttcatagaggtctgctttccaattacattctctttgttttaagtataactttgaaactcaaatataaaagcctgctacttttttttgttctaaaaagacagatgtggactaggcacctgtactgtgaaaccagaatagagaagctgttgggcagatttgaagaggattgagtaatatagagaatgtcttgagatatttgtgaagcttttattgctttgttgcaattgttgtctagaaacatgggctttttctgttttttctcctattccaggagaggagggcgcatcacttcagaaaaggaagagcagtgctcaaaagtgttggatccggagctactaacttcagcctgctgaagcaggctggagacgtggaggagaaccctggacctatgctcgagggagtgcaggtggagactatctccccaggagacgggcgcaccttccccaagcgcggccagacctgcgtggtgcactacaccgggatgcttgaagatggaaagaaagttgattcctcccgggacagaaacaagccctttaagtttatgcttggcaagcaggaggtgatccgaggctgggaagaaggggttgcccagatgagtgtgggtcagagagccaaactgactatatctccagattatgcctatggtgccactgggcacccaggcatcatcccaccacatgccactctcgtcttcgatgtggagcttctaaaactggaatctggcggtggttccggagtcgacggtgtctctgtgaattgcagaccagctaggatgcatgctagtgcatgccaggtgtaccagctgcgagcagacccttgtgggcactgcctgatcttcaacaatgtcagcttcagcagagactctgatctgtcgactcgagctggctctgacatagactgtgagaagctggagaagcgtttcaggtccctgtgcttccacgtccggaccctgcggaacctcaaagctcaggaaattgatgtggagctgcggaagctggcgcggctcgaccacagtgccctggactgctgcctcgtggtcatcctctcccatggttgccagacaagccatattcagtttcccggagggatttatggaacagatggcaaaatcattccaatcgaaaggattgtgaactatttcaatgggtcccagtgcccgagtttgagaggaaaacccaaactcttcttcatccaggcctgtggaggagaacaaaaggaccaaggatttgaggtggattgtgaatcaccccaagatgaaacttgccgacgttccatagagtcggatgcgattcctttccaggctccatcagggaatgaggacgagccagacgccgtcgccagtttgcccactcctggtgacatcttggtgtcctattcaacttttccaggttttgtgtcctggagggacaaggtgagtggctcgtggtacgtggaaaccttggacagcgtactggaacattacgcccgttctgaagacctgcttaccatgctacttcgggtgtcagacatcgtatccaccaaggggaggtacaagcagatcccgggctgtttcaacttccttcgtaaaaaattcttcttcctgtgcaaggtcgactatccgtacgacgtaccagactacgcactcgacggatccggagagggcagaggaagtctgctaacatgcggtgacgtcgaggagaatcctggacctatggtgagcaagggcgaggagctgttcaccggggtggtgcccatcctggtcgagctggacggcgacgtaaacggccacaagttcagcgtgtccggcgagggcgagggcgatgccacctacggcaagctgaccctgaagttcatctgcaccaccggcaagctgcccgtgccctggcccaccctcgtgaccaccctgacctacggcgtgcagtgcttcagccgctaccccgaccacatgaagcagcacgacttcttcaagtccgccatgcccgaaggctacgtccaggagcgcaccatcttcttcaaggacgacggcaactacaagacccgcgccgaggtgaagttcgagggcgacaccctggtgaaccgcatcgagctgaagggcatcgacttcaaggaggacggcaacatcctggggcacaagctggagtacaactacaacagccacaacgtctatatcatggccgacaagcagaagaacggcatcaaggtgaacttcaagatccgccacaacatcgaggacggcagcgtgcagctcgccgaccactaccagcagaacacccccatcggcgacggccccgtgctgctgcccgacaaccactacctgagcacccagtccgccctgagcaaagaccccaacgagaagcgcgatcacatggtcctgctggagttcgtgaccgccgccgggatcactctcggcatggacgagctgtacaagtgatgaacaaagactttgaagtacataaatgtattactttgatgttaatacagttcagtttagtaagatgtgtagtaaaaagtgtaaccttgttcaaaaagttgcttcaagttgatgtttgtgttctgttttacctgttccagaatagctatttttgcttgagaagtttgaagttgtaagagttgaaatatttccaggttttattactagcttgcatgcttttcctgctaactaactgaaatgctaatcttaaggaatttatatggggaaggggaaaaaagaaaaacactttgtttggtacgtgtggattttcttctgagctttaaggtacagtttgttgcatgttaaaatttagttcttattaaaccacaactttaagttactaacgtcaaccagttacctcttgcagttcaaaagttgaagcagttccttgtccaagatggagtattttaaaactgagctcttaatcagtggaacagaagacgtcacggtgtaactcaactgaagccctttaagtcccggttctctttagactacctaatcaatgtctttgtttgctaacgacagtttatctatgtgaatcctaaaattcctatatgtaacttaagatgcaagaatgtaattagttacattggctgctcagtggagtatgacttttttttttactggattaattttagcaatacctgtatcttaaaattgtgagaaaatactgcatttaaaatatgcctaactttgtgatgcaatatgttaatcaaagaatacatgtaagcatattttaataataattatgtagattttagtcatgtattttgaaacaattaaaatttttaattttgacttaccttcccagtgtgagtgacatcctaatataatacttctaaatcttaagctgctttgagaaaggcatgcagcgtatttattgaaggaattgaagatttcttaccctacataagaattccagttaggacaagtttatagcaacaaactttcacatttgctgttagttctacctgcgattttgaaggagtacaactgagaacagcactcagtcttgtatgtgtgttgggtcctagtctgattcatttttcttattactacccttatacctcagtctccaagtaaaaaaggaaataactcctcctttgtagacgtgtatatgtgaatgaatagaatggcatgtcccacttcaaatgtctagaagtagatgttggtgaaacatgcaataagagctgagttgctctgtacctggatagtgggctgtaagatgcagcacaggagtgtcccaggactgttgttcaggagtaggagtcaggggagggaggcagggcttgggggatagcaataatagttggtgccgttctccataaaattactcagaagcaatgttctggcagcataaatcgacctaaagttgttaactttttctctgctcagaccgttccctagcactaaagatgctgtgtccttaagtgtgtttccatactatccatcaccatgtttttcccaacctattgctttaatagtattg

SEQ ID NO: 5 - DNA, 5161 bp, Artificial Sequence
  Left arm-2a-iCaspase9-T2a-GFP-Right arm
cttcgtggcttggtgaagagatcttctgacctcttcatcaccccctagaattaaggctgtaatcatcatttcagccattgcttaatccactataatttctgcatgatttcagaaggctatcttgcttccttgaaactaataatacctagtttgtagtgtttagggatgtgtaaaatgtgtttatgtcaagattttagttagtctgataagaattgtggaagaattgcagctactaaaaaggcagactgggtagcacttcccaccttactcagatttaggagtctcaagacatgtagatgggtgaaatttattattcttttctctgcttgcttttctggaaagctacctctatttggccagcagttggctctgaattcctttctttaaaggagacctgactgctctcctgtctgcctcttacacagctgtactggtgtgtcactgatagaaacgtttaccttgaaagtgacaagtgggggcgttgatacccattaacaacattaaagggaaaatttcaggaaacaagaaaactgagaggagttcagaatgaaatgtaagccctgtgacagactcacactgatggtagtagggtaactgatggagatgcatctataacaattctaacttttatttcagaagtctgtggacaggagcatacaaacagtagtatcttgtctgtttaaccctgaaaaccgtctgaggaacacctttgtatcacaagaagactacttcagggtatgtagtgaaagcaaaactaaatctctaaaaccagctgatcttaactttgttcatatacaggatgccatgaagacaaaggtttatctgtacttgcttgagattttactttttgtatgtgcattgagatgaatgactggttagctctcagttggttaatactcaatgaaaattgcagaaattgagttcagtggatttaagtgcattgatacaaggctgcataagaactgctgagcagtcagctattggatatttagagctaatcatccctcaggagcaatctgctgaaaggtaagcagattgcatcttgtaaacgagagagcagagttaaacgtttgtggtctttgctccacttaagtacccacagtggatgtctatctgtacttttggttaaaaaatagataatttctacaacagactgtagttaggtcagtacctggtcatcaggtattaatggaaagctttttgctgtgcattcaatcttcatagaggtctgctttccaattacattctctttgttttaagtataactttgaaactcaaatataaaagcctgctacttttttttgttctaaaaagacagatgtggactaggcacctgtactgtgaaaccagaatagagaagctgttgggcagatttgaagaggattgagtaatatagagaatgtcttgagatatttgtgaagcttttattgctttgttgcaattgttgtctagaaacatgggctttttctgttttttctcctattccaggagaggagggcgcatcacttcagaaaaggaagagcagtgctcaaaagtgttggatccggagctactaacttcagcctgctgaagcaggctggagacgtggaggagaaccctggacctatgctcgagggagtgcaggtggagactatctccccaggagacgggcgcaccttccccaagcgcggccagacctgcgtggtgcactacaccgggatgcttgaagatggaaagaaagttgattcctcccgggacagaaacaagccctttaagtttatgctaggcaagcaggaggtgatccgaggctgggaagaaggggttgcccagatgagtgtgggtcagagagccaaactgactatatctccagattatgcctatggtgccactgggcacccaggcatcatcccaccacatgccactctcgtcttcgatgtggagcttctaaaactggaatctggcggtggttccggagtcgacggatttggtgatgtcggtgctcttgagagtttgaggggaaatgcagatttggcttacatcctgagcatggagccctgtggccactgcctcattatcaacaatgtgaacttctgccgtgagtccgggctccgcacccgcactggctccaacatcgactgtgagaagttgcggcgtcgcttctcctcgctgcatttcatggtggaggtgaagggcgacctgactgccaagaaaatggtgctggctttgctggagctggcgcggcaggaccacggtgctctggactgctgcgtggtggtcattctctctcacggctgtcaggccagccacctgcagttcccaggggctgtctacggcacagatggatgccctgtgtcggtcgagaagattgtgaacatcttcaatgggaccagctgccccagcctgggagggaagcccaagctctttttcatccaggcctgtggtggggagcagaaagaccatgggtttgaggtggcctccacttcccctgaagacgagtcccctggcagtaaccccgagccagatgccaccccgttccaggaaggtttgaggaccttcgaccagctggacgccatatctagtttgcccacacccagtgacatctttgtgtcctactctactttcccaggttttgtttcctggagggaccccaagagtggctcctggtacgttgagaccctggacgacatctttgagcagtgggctcactctgaagacctgcagtccctcctgcttagggtcgctaatgctgtttcggtgaaagggatttataaacagatgcctggttgctttaatttcctccggaaaaaacttttctttaaaacatcagtcgactatccgtacgacgtaccagactacgcactcgacctcgacggatccggagagggcagaggaagtctgctaacatgcggtgacgtcgaggagaatcctggacctatggtgagcaagggcgaggagctgttcaccggggtggtgcccatcctggtcgagctggacggcgacgtaaacggccacaagttcagcgtgtccggcgagggcgagggcgatgccacctacggcaagctgaccctgaagttcatctgcaccaccggcaagctgcccgtgccctggcccaccctcgtgaccaccctgacctacggcgtgcagtgcttcagccgctaccccgaccacatgaagcagcacgacttcttcaagtccgccatgcccgaaggctacgtccaggagcgcaccatcttcttcaaggacgacggcaactacaagacccgcgccgaggtgaagttcgagggcgacaccctggtgaaccgcatcgagctgaagggcatcgacttcaaggaggacggcaacatcctggggcacaagctggagtacaactacaacagccacaacgtctatatcatggccgacaagcagaagaacggcatcaaggtgaacttcaagatccgccacaacatcgaggacggcagcgtgcagctcgccgaccactaccagcagaacacccccatcggcgacggccccgtgctgctgcccgacaaccactacctgagcacccagtccgccctgagcaaagaccccaacgagaagcgcgatcacatggtcctgctggagttcgtgaccgccgccgggatcactctcggcatggacgagctgtacaagtgatgaacaaagactttgaagtacataaatgtattactttgatgttaatacagttcagtttagtaagatgtgtagtaaaaagtgtaaccttgttcaaaaagttgcttcaagttgatgtttgtgttctgttttacctgttccagaatagctatttttgcttgagaagtttgaagttgtaagagttgaaatatttccaggttttattactagcttgcatgcttttcctgctaactaactgaaatgctaatcttaaggaatttatatggggaaggggaaaaaagaaaaacactttgtttggtacgtgtggattttcttctgagctttaaggtacagtttgttgcatgttaaaatttagttcttattaaaccacaactttaagttactaacgtcaaccagttacctcttgcagttcaaaagttgaagcagttccttgtccaagatggagtattttaaaactgagctcttaatcagtggaacagaagacgtcacggtgtaactcaactgaagccctttaagtcccggttctctttagactacctaatcaatgtctttgtttgctaacgacagtttatctatgtgaatcctaaaattcctatatgtaacttaagatgcaagaatgtaattagttacattggctgctcagtggagtatgacttttttttttactggattaattttagcaatacctgtatcttaaaattgtgagaaaatactgcatttaaaatatgcctaactttgtgatgcaatatgttaatcaaagaatacatgtaagcatattttaataataattatgtagattttagtcatgtattttgaaacaattaaaatttttaattttgacttaccttcccagtgtgagtgacatcctaatataatacttctaaatcttaagctgctttgagaaaggcatgcagcgtatttattgaaggaattgaagatttcttaccctacataagaattccagttaggacaagtttatagcaacaaactttcacatttgctgttagttctacctgcgattttgaaggagtacaactgagaacagcactcagtcttgtatgtgtgttgggtcctagtctgattcatttttcttattactacccttatacctcagtctccaagtaaaaaaggaaataactcctcctttgtagacgtgtatatgtgaatgaatagaatggcatgtcccacttcaaatgtctagaagtagatgttggtgaaacatgcaataagagctgagttgctctgtacctggatagtgggctgtaagatgcagcacaggagtgtcccaggactgttgttcaggagtaggagtcaggggagggaggcagggcttgggggatagcaataatagttggtgccgttctccataaaattactcagaagcaatgttctggcagcataaatcgacctaaagttgttaactttttctctgctcagaccgttccctagcactaaagatgctgtgtccttaagtgtgtttccatactatccatcaccatgtttttcccaacctattgctttaatagtattg

SEQ ID NO: 6 - DNA, 6579 bp, Artificial Sequence
  Left arm-GFP-2a-iCaspase9-T2a-Right arm
tttttttctttgagatgagtatcttattgcagctctgtgcataccccttgaaaatccgtaggtgatgtatttatgttgactgaaaatggagtcattcaaaaattgatgacttcttccttttctctttttaatctcgaaacctgttctcagattcctttatcagaacaaaaagcacggctgcatgtttttcaccgttcacacgactgtgtttagccagcgtatctaaatgcataacatgatttgccataacttgagcctgccataatcagagcctcattttgaaagctgtcatggtctgaaacatagcatgggtaagatgattttcaccttgatgatgcatgtttaactcatttcaacgagaggtcaaatccatccaaaaatgctaaatctatcaaccagttttcatgttcaagttctggcacaaattttcgttctgactccatacgtgattagatttcattttgcaaatcatgaaaactattgccaaaacatacaattttaagtcagcagttttactgcccaaatttgcacaagcacatgtaacgtgacagacaaaaacccactggacagagacaaaatactgggtttggccagtatggtttggctaagccacgtttttcagggcaagaattgcctcacctttttttatattggaatcaaattctcaagtgtaacagcctggcgccatctcagctgccattaagtagcatgtgctgcaacaagatgtctaccacacactctgctctgggtggtgggggcacaccagtgtggacggcaaccatgacacaagcatagagtcttggcagaggtccattgggtgcatttatagtggttcacactggggggttatcacagaatcatggaggttggaaggtacctccgggggtcatcaaatccaaccacttgacaaagcaggttccctaaagtagattgctcaagaacagtcacagcactgctgctcacagaaaatctctagttggtaaggttacctttttttttgttgtcgctcccagttaaaccaaggtgggaacacatccttttcatagttgtattgtagggatgtttatagctattgctagggaaaactgaacagcgtgcaaggaagtcagcactgacacagctttcccacgtgagagagctatttcaaagcaagatcagcacatatcccaatctgtacttcctcaaacacagcccaaaaccgatagcaaggccaagcagcagcactgctccttcaaggaaactgctgcataatctgaatttcagacggcaggaggaaacaaggcagcagactgatgacctaccaccctgagtctcagctacatgcgatccgagccactccaactctgcttcctgcagcccttccttcacgctcatcttttgcaccttaggcactcttataattcaagtactttgtggctttgggatatttgaagagcttggtcagttagtcacaagtctggccacgtgctatcatattagtttgaaaagcaatggagacaccatctgctgatgctcaaagtggttacaaccaaaacacaaaaaagcagagctgtgggaagaattcaacattttgattatgcaagaagctagtcccagccttgaaatccaccatctgcatcatgaaagacctaagtagttaaagccacagcagacatacagcttctatttccttaccttcttcatcattaactacaggtcttggaagatttttgctgggaaaaagcttttattgcaagaactgtaatttattaacagggaaacatgaaataaatgtgtaaattctcctgcactcccactgtcattaaaaacggctttaagaaagagtattcagtaactgcctgcattgtgttgtgactttctactctgtgacacacagccttctgggcaaagcacatattctgccatgcatgtgggtcgtgccttggaaaatgggaacccacattcactgagggcctcttgatgagctttccccttgagaacagcgaggtctcatggatatcttctcttctccaagccaaataagcccagatccctcagctttccttcatggagaggctccagccctctgatcatgcctgcagcccttctctggacctgctccagcagccccacacgctcctcatgctgggaccccagatctgcacatggtattgcacatggggcctcacaacggcagagctgagagggacaattccctccctcagcctttaattctgcacgtacttaattttgtctgtattttttttgcaatagaatagcctgcatgctagttgctgtgtcgcacagctgaattcactaggttcctgtgaaacaaagggcaatcccacagccactgtagcacgtgaggagccacacaggtgctctaattcctacaggacaggcctagggacagagcggccctaggactgccctcccgcacctcctagcttcaccttttgcccgcgatctttaagtaccctgaagcataaacagggaaagcgccgcccgcagcctcaccctgcttcccgcccaacgcggcaccgcccaggccgcagccgcccactaagagcactagcgccaccttctcaccccacccccaccacgcgttcctagcggccctgagagctgctgcgcatgcgccgcctgacgattcgccctcccattggctggcggtcgaagcacggcgggggcacgcggtggcggctatataaggcgtctcggaagacggcgccatgctatttggagcggagagtgaaagttacagttcctggtgctggtagggagtgtggcgcggagcggagcgctgcggctcatcggaaccacaatggagccatagcagagccgggcgtgggggcaagggcagtgcgtgctggggagggctccgtcgcgtggccacgtcgcgagagccgtcgggatggtggcgtcagggcggggggtgctgctaacgtgctcctggtcctgcaggtgggctgctggcattcgccatggtgagcaagggcgaggagctgttcaccggggtggtgcccatcctggtcgagctggacggcgacgtaaacggccacaagttcagcgtgtccggcgagggcgagggcgatgccacctacggcaagctgaccctgaagttcatctgcaccaccggcaagctgcccgtgccctggcccaccctcgtgaccaccctgacctacggcgtgcagtgcttcagccgctaccccgaccacatgaagcagcacgacttcttcaagtccgccatgcccgaaggctacgtccaggagcgcaccatcttcttcaaggacgacggcaactacaagacccgcgccgaggtgaagttcgagggcgacaccctggtgaaccgcatcgagctgaagggcatcgacttcaaggaggacggcaacatcctggggcacaagctggagtacaactacaacagccacaacgtctatatcatggccgacaagcagaagaacggcatcaaggtgaacttcaagatccgccacaacatcgaggacggcagcgtgcagctcgccgaccactaccagcagaacacccccatcggcgacggccccgtgctgctgcccgacaaccactacctgagcacccagtccgccctgagcaaagaccccaacgagaagcgcgatcacatggtcctgctggagttcgtgaccgccgccgggatcactctcggcatggacgagctgtacaagggatccggagctactaacttcagcctgctgaagcaggctggagacgtggaggagaaccctggacctatgctcgagggagtgcaggtggagactatctccccaggagacgggcgcaccttccccaagcgcggccagacctgcgtggtgcactacaccgggatgcttgaagatggaaagaaagttgattcctcccgggacagaaacaagccctttaagtttatgctaggcaagcaggaggtgatccgaggctgggaagaaggggttgcccagatgagtgtgggtcagagagccaaactgactatatctccagattatgcctatggtgccactgggcacccaggcatcatcccaccacatgccactctcgtcttcgatgtggagcttctaaaactggaatctggcggtggatccggagtcgacggatttggtgatgtcggtgctcttgagagtttgaggggaaatgcagatttggcttacatcctgagcatggagccctgtggccactgcctcattatcaacaatgtgaacttctgccgtgagtccgggctccgcacccgcactggctccaacatcgactgtgagaagttgcggcgtcgcttctcctcgctgcatttcatggtggaggtgaagggcgacctgactgccaagaaaatggtgctggctttgctggagctggcgcggcaggaccacggtgctctggactgctgcgtggtggtcattctctctcacggctgtcaggccagccacctgcagttcccaggggctgtctacggcacagatggatgccctgtgtcggtcgagaagattgtgaacatcttcaatgggaccagctgccccagcctgggagggaagcccaagctctttttcatccaggcctgtggtggggagcagaaagaccatgggtttgaggtggcctccacttcccctgaagacgagtcccctggcagtaaccccgagccagatgccaccccgttccaggaaggtttgaggaccttcgaccagctggacgccatatctagtttgcccacacccagtgacatctttgtgtcctactctactttcccaggttttgtttcctggagggaccccaagagtggctcctggtacgttgagaccctggacgacatctttgagcagtgggctcactctgaagacctgcagtccctcctgcttagggtcgctaatgctgtttcggtgaaagggatttataaacagatgcctggttgctttaatttcctccggaaaaaacttttctttaaaacatcagtcgactatccgtacgacgtaccagactacgcactcgacctcgacggatccggagagggcagaggaagtctgctaacatgcggtgacgtcgaggagaatcctggacctatggaggaggattgggataccgaactcgagcaggaggcggcagcggcttcccaggggcgttctgaggagcaggcgtggatggtgagctgtgtccaggggagggcggtgcggcagggagcggggcactgggatggcccggtctgggaaggggaggccgagaggccttcgcagtgcttcctgcagctccccgagcagtgcgaagaaggaggtgccgggctctgctgtgggagccgaaggcacggagctgcctggggagggaatggctgtgtgcctgaggtgccagagaccggcaagggctgtacagagaggcaacggttttgtgtacaaatcatttgtatgggaaaccacaaaatcttgaagctttattacatggcagcgaaatactttggtgtgaagtaaaggataagatagaggagtgtaatgagagacagctaaataatattttactacttgtgggatgagtgaatatcaggaggaactgctgtaaatttcaggaggacctgttgtgaatcttcagtagttggcgccgctcttacacatcttacagatgccccttgagcaaagggggataaggagagatgaacgggttatccaaacaggtgatgagctaaaagtacagttgcctaaagaagtagtagcatgtgctatcagaatgataattttgttagtttggggttagtttcctgtagtggtagatagccacaacaagaaaaccgcttaagtttttgtaaaacaaaaaaagcacgatccagaagtaaaaaatatgggtagttttttttgatgttcctctctcacctggtgctttggcatactaatatgtgtctaattgtattaaacaggagaaatttaaacctaggctttgctggaaataaaatgttacaatgctacaatgtgaaaagtaggtgctattctgaactgttttgggtggagtatctgaatctttgaataatttaagagggactgacatatttaaaatacttaaggataatctgtagccatgctgtaaaagaacaacagaaatgcagttgggaaggtgatggaaatagttttattcatgttactggtggtctgaaacctttctaagcttaaactgtagaaaaaaattgcttcaaaagattgcactattactttgggcgacaaatgtttttaattggttttaagtgtttgttagcaaagtgaagttgatgccaccataagtctgacaggaggcaagataaacttgtcttcatactgcttgtgtataacttggttttgatgacatttgtgtgtgaacattatgcacttcagtgtagcgaagtttaagaaactttgaacagaataacttgaaagagtgtgcacatgggtgcagaagtcactttatttcagttgggagacttagcacctaaatgcactgttagttcacatacactttgcttggcctgaaggtaacattgtgatgtcgctttttttccctgtaggctaactctggcagaccaaacagcccatccctccgcttctccagcagaccaagcagccccttgtctgg

SEQ ID NO: 7 - DNA, 75 bp, Artificial Sequence
  forward primer
cggtgacgtcgaggagaatcctggacctatggaggaggattgggataccgaactcgagcaggaggcggcagcggc

SEQ ID NO: 8 - DNA, 47 bp, Artificial Sequence
  reverse primer
gaaatccagcttccagttcccacctggccagacaaggggctgcttgg

SEQ ID NO: 9 - DNA, 41 bp, Artificial Sequence
  forward primer
ggtgggctgctggcattcgccatggtgagcaagggcgagga

SEQ ID NO: 10 - DNA, 76 bp, Artificial Sequence
  reverse primer
gattctcctcgacgtcaccgcatgttagcagacttcctctgccctctccggatcccttgtacagctcgtccatgcc

SEQ ID NO: 11 - DNA, 57 bp, Artificial Sequence
  forward primer
tctcccatatggtcgacctgcaggcggccgcgaattcactagtgattcttcgtggtt

SEQ ID NO: 12 - DNA, 48 bp, Artificial Sequence
  reverse primer
aggctgaagttagtagctccggatccaacacttttgagcactgctctt

SEQ ID NO: 13 - DNA, 107 bp, Artificial Sequence
  forward primer
cagaacatcaccctgaccgaggtgggatccggagagggcagaggaagtctgctaacatgcggtgacgtcgaggagaatcctggacctatggtgagcaagggcgagga

SEQ ID NO: 14 - DNA, 22 bp, Artificial Sequence
  reverse primer
cttgtacagctcgtccatgccg

SEQ ID NO: 15 - DNA, 94 bp, Artificial Sequence
  forward primer
tctcggcatggacgagctgtacaagtgatgaacaaagactttgaagtacataaatgtattactttgatgttaatacagttcagtttagtaagat

SEQ ID NO: 16 - DNA, 55 bp, Artificial Sequence
  reverse primer
ctcttcgaaatccagcttccagttcccacctggcaatactattaaagcaataggt

SEQ ID NO: 17 - DNA, 20 bp, Artificial Sequence
  guide sequence
ggtcctattccaggagagga

SEQ ID NO: 18 - DNA, 20 bp, Artificial Sequence
  guide sequence
ggcttactaaactgaactgt